European Patent Application EP 4 538 368 A1, published April 16, 2025. Title: 热稳定性改善的葡萄糖氧化酶GoxM10突变体E361P及其衍生突变体和应用. Applicant: 中国农业科学院北京畜牧兽医研究所. The sequence listing filed with the application follows.

SEQUENCE LISTING (41 sequences)

SEQ ID NO: 1 - protein, 581 aa, synthetic construct
GIEASLLTDPKEVAGRTVDYIIAGGGLTGLVVAARLTENPDITVLVIESGSYESDRGPIIEDLNAYGKIFGSSVDHAYETVCLATNNRTALIRAGNGLGGSTLVNGGTWTRPHKAQVDSWETVFGNEGWNWDSVAAYSLQAERARAPNAKQIAAGHYFNASCHGINGTVHAGPRDTGDDYSPIVKALMSAVEDRGVPTKKDLGCGDPHGVSMFPNTLHEDQVRSDAAREWLLPNYQRPNLQVLTGQYVGKVLLSQNATTPRAVGVEFGTHKGNFHNVTAKHEVLLAAGSAVSPTILEYSGIGMKSILEPLGIKTVVDLPVGLNLQDQTTSTVRSRITSAGAGQGQAAWFATFNETFGDYTEKAHELLNTKLEQWAEEAVARGGFHNTTALLIQYENYRDWIVKDNVAYSELFLDTAGEASFDVWDLLPFTRGYVHILDKDPYLRHFAYDPQYFLNELDLLGQAAATQLARNISNSGAMQTYFAGETIPGDNLAYDADLRAWVEYIPYHFRPNYHGVGTCSMMPKEMGGVVDNAARVYGVQGLRVIDGSIPPTQMSSHVMTVFYAMALKIADAVLADYASMQ

SEQ ID NO: 2 - protein, 581 aa, synthetic construct
GIEASLLTDPKEVAGRTVDYIIAGGGLTGLVVAARLTENPDITVLVIESGSYESDRGPIIEDLNAYGKIFGSSVDHAYETVCLATNNRTALIRAGNGLGGSTLVNGGTWTRPHKAQVDSWETVFGNEGWNWDSVAAYSLQAERARAPNAKQIAAGHYFNASCHGINGTVHAGPRDTGDDYSPIVKALMSAVEDRGVPTKKDLCCGDPHGVSMFPNTLHEDQVRSDAAREWLLPNYQRPNLSVLTGQYVGKVLLSQNATTPRAVGVEFGTHKGNFHNVTAKHEVLLAAGSAVSPTILEYSGIGMKSILEPLGIKTVVDLPVGLNLQDQTTSTVRSRITSAGAGQGQAAWFATFNETFGDYTEKAHELLNTKLEQWAEEAVARGGFHNTTALLIQYENYRDWIVKDNVAYSELFLDTAGEASFDVWDLLPFTRGYVHILDKDPYLRHFAYDPQYFLNELDLLGQAAATQLARNISNSGAMQTYFAGETIPGDNLAYDADLRAWVEYIPYHFRPNYHGVGTCSMMPKEMGGVVDNAARVYGVQGLRVIDGSIPPTQMSSHVMTVFYAMALKIADAVLADYASMQ

SEQ ID NO: 3 - DNA, 1746 bp, synthetic construct
  source 1..1746: mol_type = other DNA
ggtattgaggcttccttgttgactgacccaaaggaggtcgccggtagaactgttgactacatcattgctggtggtggattgactggtttggttgtcgctgccagattgactgagaacccagacatcaccgttttggtcattgagtccggttcttacgaatctgatagaggtcctatcattgaagacttgaacgcttacggtaaaatcttcggatcttccgttgaccacgcttacgagactgtctgccttgccactaacaatagaaccgctttgattagagctggtaacggtttgggtggttctactttggttaacggaggtacttggaccagaccacacaaggctcaagttgactcttgggagaccgtcttcggtaacgaaggttggaattgggattctgtcgcagcttactccttgcaggccgagagagcccgtgctccaaacgctaagcaaatcgccgcaggtcactacttcaacgcctcctgtcacggtattaacggaactgttcacgctggtccaagagacaccggtgacgattactctcctatcgtcaaggccttgatgtccgctgttgaagacagaggtgtcccaactaagaaggacttgtgttgcggagacccacatggtgtttctatgttccctaacaccttgcacgaggaccaagtcagatccgatgctgcccgtgaatggttgcttccaaactaccaaagacctaacttgcaggttttgaccggtcaatacgttggtaaggtccttttgtctcaaaacgccactaccccaagagctgttggtgtcgagttcggaactcacaagggtaactttcacaatgttaccgctaaacacgaagtccttttggcagctggttccgctgtttctccaactatcttggagtactctggtatcggaatgaagtccattttggaaccacttggtattaagaccgtcgttgacttgcctgttggtctgaacttgcaagaccagactacctctactgtcagatcccgtattacctccgccggtgctggacagggtcaggctgcctggtttgctactttcaacgagaccttcggtgactacactgagaaggctcacgaattgcttaacaccaaattggaacaatgggctgaggaagccgttgctagaggtggtttccacaacactaccgctcttttgatccaatacgagaactacagagactggattgttaaggataacgtcgcttactctgaattgttcttggacactgccggtgaggcttccttcgacgtctgggacttgctgccattcactagaggatacgttcacatcttggacaaggacccatacttgagacacttcgcttacgatcctcaatacttcttgaacgagttggacttgcttggtcaggctgccgctactcaattggctagaaacatctctaactccggtgccatgcaaacttactttgctggtgaaaccattccaggtgacaacttggcctacgatgctgacttgagagcttgggttgaatacattccataccacttcagacctaactaccatggtgtcggaacctgttctatgatgccaaaggagatgggtggtgtcgttgacaacgccgctagagtttacggtgtccagggattgagagttatcgacggttctatcccacctactcaaatgtcctctcacgttatgaccgtcttctacgctatggctttgaagatcgcagacgctgttttggctgactacgcctccatgcaataa

SEQ ID NO: 4 - protein, 581 aa, synthetic construct
GIEASLLTDPKEVAGRTVDYIIAGGGLTGLVVAARLTENPDITVLVIESGSYESDRGPIIEDLNAYGKIFGSSVDHAYETVCLATNNRTALIRAGNGLGGSTLVNGGTWTRPHKAQVDSWETVFGNEGWNWDSVAAYSLQAERARAPNAKQIAAGHYFNASCHGINGTVHAGPRDTGDDYSPIVKALMSAVEDRGVPTKKDLGCGDPHGVSMFPNTLHPDQVRSDAAREWLLPNYQRPNLSVLTGQYVGKVLLSQNATTPRAVGVEFGTHKGNFHNVTAKHEVLLAAGSAVSPTILEYSGIGMKSILEPLGIKTVVDLPVGLNLQDQTTSTVRSRITSAGAGQGQAAWFATFNETFGDYTEKAHELLNTKLEQWAEEAVARGGFHNTTALLIQYENYRDWIVKDNVAYSELFLDTAGEASFDVWDLLPFTRGYVHILDKDPYLRHFAYDPQYFLNELDLLGQAAATQLARNISNSGAMQTYFAGETIPGDNLAYDADLRAWVEYIPYHFRPNYHGVGTCSMMPKEMGGVVDNAARVYGVQGLRVIDGSIPPTQMSSHVMTVFYAMALKIADAVLADYASMQ

SEQ ID NO: 5 - DNA, 1746 bp, synthetic construct
  source 1..1746: mol_type = other DNA
ggtattgaggcttccttgttgactgacccaaaggaggtcgccggtagaactgttgactacatcattgctggtggtggattgactggtttggttgtcgctgccagattgactgagaacccagacatcaccgttttggtcattgagtccggttcttacgaatctgatagaggtcctatcattgaagacttgaacgcttacggtaaaatcttcggatcttccgttgaccacgcttacgagactgtctgccttgccactaacaatagaaccgctttgattagagctggtaacggtttgggtggttctactttggttaacggaggtacttggaccagaccacacaaggctcaagttgactcttgggagaccgtcttcggtaacgaaggttggaattgggattctgtcgcagcttactccttgcaggccgagagagcccgtgctccaaacgctaagcaaatcgccgcaggtcactacttcaacgcctcctgtcacggtattaacggaactgttcacgctggtccaagagacaccggtgacgattactctcctatcgtcaaggccttgatgtccgctgttgaagacagaggtgtcccaactaagaaggacttgggttgcggagacccacatggtgtttctatgttccctaacaccttgcacccagaccaagtcagatccgatgctgcccgtgaatggttgcttccaaactaccaaagacctaacttgcaggttttgaccggtcaatacgttggtaaggtccttttgtctcaaaacgccactaccccaagagctgttggtgtcgagttcggaactcacaagggtaactttcacaatgttaccgctaaacacgaagtccttttggcagctggttccgctgtttctccaactatcttggagtactctggtatcggaatgaagtccattttggaaccacttggtattaagaccgtcgttgacttgcctgttggtctgaacttgcaagaccagactacctctactgtcagatcccgtattacctccgccggtgctggacagggtcaggctgcctggtttgctactttcaacgagaccttcggtgactacactgagaaggctcacgaattgcttaacaccaaattggaacaatgggctgaggaagccgttgctagaggtggtttccacaacactaccgctcttttgatccaatacgagaactacagagactggattgttaaggataacgtcgcttactctgaattgttcttggacactgccggtgaggcttccttcgacgtctgggacttgctgccattcactagaggatacgttcacatcttggacaaggacccatacttgagacacttcgcttacgatcctcaatacttcttgaacgagttggacttgcttggtcaggctgccgctactcaattggctagaaacatctctaactccggtgccatgcaaacttactttgctggtgaaaccattccaggtgacaacttggcctacgatgctgacttgagagcttgggttgaatacattccataccacttcagacctaactaccatggtgtcggaacctgttctatgatgccaaaggagatgggtggtgtcgttgacaacgccgctagagtttacggtgtccagggattgagagttatcgacggttctatcccacctactcaaatgtcctctcacgttatgaccgtcttctacgctatggctttgaagatcgcagacgctgttttggctgactacgcctccatgcaataa

SEQ ID NO: 6 - protein, 581 aa, synthetic construct; identical to SEQ ID NO: 2

SEQ ID NO: 7 - DNA, 1746 bp, synthetic construct
  source 1..1746: mol_type = other DNA
ggtattgaggcttccttgttgactgacccaaaggaggtcgccggtagaactgttgactacatcattgctggtggtggattgactggtttggttgtcgctgccagattgactgagaacccagacatcaccgttttggtcattgagtccggttcttacgaatctgatagaggtcctatcattgaagacttgaacgcttacggtaaaatcttcggatcttccgttgaccacgcttacgagactgtctgccttgccactaacaatagaaccgctttgattagagctggtaacggtttgggtggttctactttggttaacggaggtacttggaccagaccacacaaggctcaagttgactcttgggagaccgtcttcggtaacgaaggttggaattgggattctgtcgcagcttactccttgcaggccgagagagcccgtgctccaaacgctaagcaaatcgccgcaggtcactacttcaacgcctcctgtcacggtattaacggaactgttcacgctggtccaagagacaccggtgacgattactctcctatcgtcaaggccttgatgtccgctgttgaagacagaggtgtcccaactaagaaggacttgggttgcggagacccacatggtgtttctatgttccctaacaccttgcacgaggaccaagtcagatccgatgctgcccgtgaatggttgcttccaaactaccaaagacctaacttgcaggttttgaccggtcaatacgttggtaaggtccttttgtctcaaaacgccactaccccaagagctgttggtgtcgagttcggaactcacaagggtaactttcacaatgttaccgctaaacacgaagtccttttggcagctggttccgctgtttctccaactatcttggagtactctggtatcggaatgaagtccattttggaaccacttggtattaagaccgtcgttgacttgcctgttggtctgaacttgcaagaccagactacctctactgtcagatcccgtattaccccagccggtgctggacagggtcaggctgcctggtttgctactttcaacgagaccttcggtgactacactgagaaggctcacgaattgcttaacaccaaattggaacaatgggctgaggaagccgttgctagaggtggtttccacaacactaccgctcttttgatccaatacgagaactacagagactggattgttaaggataacgtcgcttactctgaattgttcttggacactgccggtgaggcttccttcgacgtctgggacttgctgccattcactagaggatacgttcacatcttggacaaggacccatacttgagacacttcgcttacgatcctcaatacttcttgaacgagttggacttgcttggtcaggctgccgctactcaattggctagaaacatctctaactccggtgccatgcaaacttactttgctggtgaaaccattccaggtgacaacttggcctacgatgctgacttgagagcttgggttgaatacattccataccacttcagacctaactaccatggtgtcggaacctgttctatgatgccaaaggagatgggtggtgtcgttgacaacgccgctagagtttacggtgtccagggattgagagttatcgacggttctatcccacctactcaaatgtcctctcacgttatgaccgtcttctacgctatggctttgaagatcgcagacgctgttttggctgactacgcctccatgcaataa

SEQ ID NO: 8 - protein, 581 aa, synthetic construct
GIEASLLTDPKEVAGRTVDYIIAGGGLTGLVVAARLTENPDITVLVIESGSYESDRGPIIEDLNAYGKIFGSSVDHAYETVCLATNNRTALIRAGNGLGGSTLVNGGTWTRPHKAQVDSWETVFGNEGWNWDSVAAYSLQAERARAPNAKQIAAGHYFNASCHGINGTVHAGPRDTGDDYSPIVKALMSAVEDRGVPTKKDLGCGDPHGVSMFPNTLHEDQVRSDAAREWLLPNYQRPNLSVLTGQYVGKVLLSQNATTPRAVGVEFGTHKGNFHNVTAKHEVLLAAGSAVSPTILEYSGIGMKSILEPLGIKTVVDLPVGLNLQDQTTSTVRSRITSAGAGQGQAAWFATFNETFGDYTPKAHELLNTKLEQWAEEAVARGGFHNTTALLIQYENYRDWIVKDNVAYSELFLDTAGEASFDVWDLLPFTRGYVHILDKDPYLRHFAYDPQYFLNELDLLGQAAATQLARNISNSGAMQTYFAGETIPGDNLAYDADLRAWVEYIPYHFRPNYHGVGTCSMMPKEMGGVVDNAARVYGVQGLRVIDGSIPPTQMSSHVMTVFYAMALKIADAVLADYASMQ

SEQ ID NO: 9 - DNA, 1746 bp, synthetic construct
  source 1..1746: mol_type = other DNA
ggtattgaggcttccttgttgactgacccaaaggaggtcgccggtagaactgttgactacatcattgctggtggtggattgactggtttggttgtcgctgccagattgactgagaacccagacatcaccgttttggtcattgagtccggttcttacgaatctgatagaggtcctatcattgaagacttgaacgcttacggtaaaatcttcggatcttccgttgaccacgcttacgagactgtctgccttgccactaacaatagaaccgctttgattagagctggtaacggtttgggtggttctactttggttaacggaggtacttggaccagaccacacaaggctcaagttgactcttgggagaccgtcttcggtaacgaaggttggaattgggattctgtcgcagcttactccttgcaggccgagagagcccgtgctccaaacgctaagcaaatcgccgcaggtcactacttcaacgcctcctgtcacggtattaacggaactgttcacgctggtccaagagacaccggtgacgattactctcctatcgtcaaggccttgatgtccgctgttgaagacagaggtgtcccaactaagaaggacttgggttgcggagacccacatggtgtttctatgttccctaacaccttgcacgaggaccaagtcagatccgatgctgcccgtgaatggttgcttccaaactaccaaagacctaacttgcaggttttgaccggtcaatacgttggtaaggtccttttgtctcaaaacgccactaccccaagagctgttggtgtcgagttcggaactcacaagggtaactttcacaatgttaccgctaaacacgaagtccttttggcagctggttccgctgtttctccaactatcttggagtactctggtatcggaatgaagtccattttggaaccacttggtattaagaccgtcgttgacttgcctgttggtctgaacttgcaagaccagactacctctactgtcagatcccgtattacctccgccggtgctggacagggtcaggctgcctggtttgctactttcaacgagaccttcggtgactacactccaaaggctcacgaattgcttaacaccaaattggaacaatgggctgaggaagccgttgctagaggtggtttccacaacactaccgctcttttgatccaatacgagaactacagagactggattgttaaggataacgtcgcttactctgaattgttcttggacactgccggtgaggcttccttcgacgtctgggacttgctgccattcactagaggatacgttcacatcttggacaaggacccatacttgagacacttcgcttacgatcctcaatacttcttgaacgagttggacttgcttggtcaggctgccgctactcaattggctagaaacatctctaactccggtgccatgcaaacttactttgctggtgaaaccattccaggtgacaacttggcctacgatgctgacttgagagcttgggttgaatacattccataccacttcagacctaactaccatggtgtcggaacctgttctatgatgccaaaggagatgggtggtgtcgttgacaacgccgctagagtttacggtgtccagggattgagagttatcgacggttctatcccacctactcaaatgtcctctcacgttatgaccgtcttctacgctatggctttgaagatcgcagacgctgttttggctgactacgcctccatgcaataa

SEQ ID NO: 10 - protein, 581 aa, synthetic construct
GIEASLLTDPKEVAGRTVDYIIAGGGLTGLVVAARLTENPDITVLVIESGSYESDRGPIIEDLNAYGKIFGSSVDHAYETVCLATNNRTALIRAGNGLGGSTLVNGGTWTRPHKAQVDSWETVFGNEGWNWDSVAAYSLQAERARAPNAKQIAAGHYFNASCHGINGTVHAGPRDTGDDYSPIVKALMSAVEDRGVPTKKDLGCGDPHGVSMFPNTLHEDQVRSDAAREWLLPNYQRPNLSVLTGQYVGKVLLSQNATTPRAVGVEFGTHKGNFHNVTAKHEVLLAAGSAVSPTILEYSGIGMKSILEPLGIKTVVDLPVGLNLQDQTTSTVRSRITSAGAGQGQAAWFATFNETFGDYTEKAHELLNTKLEQWAEEAVARGGFHNTTALLIQYENYRDWIVKDNVAYSELFLDTAGEISFDVWDLLPFTRGYVHILDKDPYLRHFAYDPQYFLNELDLLGQAAATQLARNISNSGAMQTYFAGETIPGDNLAYDADLRAWVEYIPYHFRPNYHGVGTCSMMPKEMGGVVDNAARVYGVQGLRVIDGSIPPTQMSSHVMTVFYAMALKIADAVLADYASMQ

SEQ ID NO: 11 - DNA, 1746 bp, synthetic construct
  source 1..1746: mol_type = other DNA
ggtattgaggcttccttgttgactgacccaaaggaggtcgccggtagaactgttgactacatcattgctggtggtggattgactggtttggttgtcgctgccagattgactgagaacccagacatcaccgttttggtcattgagtccggttcttacgaatctgatagaggtcctatcattgaagacttgaacgcttacggtaaaatcttcggatcttccgttgaccacgcttacgagactgtctgccttgccactaacaatagaaccgctttgattagagctggtaacggtttgggtggttctactttggttaacggaggtacttggaccagaccacacaaggctcaagttgactcttgggagaccgtcttcggtaacgaaggttggaattgggattctgtcgcagcttactccttgcaggccgagagagcccgtgctccaaacgctaagcaaatcgccgcaggtcactacttcaacgcctcctgtcacggtattaacggaactgttcacgctggtccaagagacaccggtgacgattactctcctatcgtcaaggccttgatgtccgctgttgaagacagaggtgtcccaactaagaaggacttgggttgcggagacccacatggtgtttctatgttccctaacaccttgcacgaggaccaagtcagatccgatgctgcccgtgaatggttgcttccaaactaccaaagacctaacttgcaggttttgaccggtcaatacgttggtaaggtccttttgtctcaaaacgccactaccccaagagctgttggtgtcgagttcggaactcacaagggtaactttcacaatgttaccgctaaacacgaagtccttttggcagctggttccgctgtttctccaactatcttggagtactctggtatcggaatgaagtccattttggaaccacttggtattaagaccgtcgttgacttgcctgttggtctgaacttgcaagaccagactacctctactgtcagatcccgtattacctccgccggtgctggacagggtcaggctgcctggtttgctactttcaacgagaccttcggtgactacactgagaaggctcacgaattgcttaacaccaaattggaacaatgggctgaggaagccgttgctagaggtggtttccacaacactaccgctcttttgatccaatacgagaactacagagactggattgttaaggataacgtcgcttactctgaattgttcttggacactgccggtgagatctccttcgacgtctgggacttgctgccattcactagaggatacgttcacatcttggacaaggacccatacttgagacacttcgcttacgatcctcaatacttcttgaacgagttggacttgcttggtcaggctgccgctactcaattggctagaaacatctctaactccggtgccatgcaaacttactttgctggtgaaaccattccaggtgacaacttggcctacgatgctgacttgagagcttgggttgaatacattccataccacttcagacctaactaccatggtgtcggaacctgttctatgatgccaaaggagatgggtggtgtcgttgacaacgccgctagagtttacggtgtccagggattgagagttatcgacggttctatcccacctactcaaatgtcctctcacgttatgaccgtcttctacgctatggctttgaagatcgcagacgctgttttggctgactacgcctccatgcaataa

SEQ ID NO: 12 - protein, 581 aa, synthetic construct
GIEASLLTDPKEVAGRTVDYIIAGGGLTGLVVAARLTENPDITVLVIESGSYESDRGPIIEDLNAYGKIFGSSVDHAYETVCLATNNRTALIRAGNGLGGSTLVNGGTWTRPHKAQVDSWETVFGNEGWNWDSVAAYSLQAERARAPNAKQIAAGHYFNASCHGINGTVHAGPRDTGDDYSPIVKALMSAVEDRGVPTKKDLCCGDPHGVSMFPNTLHEDQVRSDAAREWLLPNYQRPNLSVLTGQYVGKVLLSQNATTPRAVGVEFGTHKGNFHNVTAKHEVLLAAGSAVSPTILEYSGIGMKSILEPLGIKTVVDLPVGLNLQDQTTSTVRSRITSAGAGQGQAAWFATFNETFGDYTPKAHELLNTKLEQWAEEAVARGGFHNTTALLIQYENYRDWIVKDNVAYSELFLDTAGEASFDVWDLLPFTRGYVHILDKDPYLRHFAYDPQYFLNELDLLGQAAATQLARNISNSGAMQTYFAGETIPGDNLAYDADLRAWVEYIPYHFRPNYHGVGTCSMMPKEMGGVVDNAARVYGVQGLRVIDGSIPPTQMSSHVMTVFYAMALKIADAVLADYASMQ

SEQ ID NO: 13 - DNA, 1746 bp, synthetic construct
  source 1..1746: mol_type = other DNA
ggtattgaggcttccttgttgactgacccaaaggaggtcgccggtagaactgttgactacatcattgctggtggtggattgactggtttggttgtcgctgccagattgactgagaacccagacatcaccgttttggtcattgagtccggttcttacgaatctgatagaggtcctatcattgaagacttgaacgcttacggtaaaatcttcggatcttccgttgaccacgcttacgagactgtctgccttgccactaacaatagaaccgctttgattagagctggtaacggtttgggtggttctactttggttaacggaggtacttggaccagaccacacaaggctcaagttgactcttgggagaccgtcttcggtaacgaaggttggaattgggattctgtcgcagcttactccttgcaggccgagagagcccgtgctccaaacgctaagcaaatcgccgcaggtcactacttcaacgcctcctgtcacggtattaacggaactgttcacgctggtccaagagacaccggtgacgattactctcctatcgtcaaggccttgatgtccgctgttgaagacagaggtgtcccaactaagaaggacttgtgttgcggagacccacatggtgtttctatgttccctaacaccttgcacgaggaccaagtcagatccgatgctgcccgtgaatggttgcttccaaactaccaaagacctaacttgcaggttttgaccggtcaatacgttggtaaggtccttttgtctcaaaacgccactaccccaagagctgttggtgtcgagttcggaactcacaagggtaactttcacaatgttaccgctaaacacgaagtccttttggcagctggttccgctgtttctccaactatcttggagtactctggtatcggaatgaagtccattttggaaccacttggtattaagaccgtcgttgacttgcctgttggtctgaacttgcaagaccagactacctctactgtcagatcccgtattacctccgccggtgctggacagggtcaggctgcctggtttgctactttcaacgagaccttcggtgactacactccaaaggctcacgaattgcttaacaccaaattggaacaatgggctgaggaagccgttgctagaggtggtttccacaacactaccgctcttttgatccaatacgagaactacagagactggattgttaaggataacgtcgcttactctgaattgttcttggacactgccggtgaggcttccttcgacgtctgggacttgctgccattcactagaggatacgttcacatcttggacaaggacccatacttgagacacttcgcttacgatcctcaatacttcttgaacgagttggacttgcttggtcaggctgccgctactcaattggctagaaacatctctaactccggtgccatgcaaacttactttgctggtgaaaccattccaggtgacaacttggcctacgatgctgacttgagagcttgggttgaatacattccataccacttcagacctaactaccatggtgtcggaacctgttctatgatgccaaaggagatgggtggtgtcgttgacaacgccgctagagtttacggtgtccagggattgagagttatcgacggttctatcccacctactcaaatgtcctctcacgttatgaccgtcttctacgctatggctttgaagatcgcagacgctgttttggctgactacgcctccatgcaataa

SEQ ID NO: 14 - protein, 581 aa, synthetic construct
GIEASLLTDPKEVAGRTVDYIIAGGGLTGLVVAARLTENPDITVLVIESGSYESDRGPIIEDLNAYGKIFGSSVDHAYETVCLATNNRTALIRAGNGLGGSTLVNGGTWTRPHKAQVDSWETVFGNEGWNWDSVAAYSLQAERARAPNAKQIAAGHYFNASCHGINGTVHAGPRDTGDDYSPIVKALMSAVEDRGVPTKKDLGCGDPHGVSMFPNTLHPDQVRSDAAREWLLPNYQRPNLSVLTGQYVGKVLLSQNATTPRAVGVEFGTHKGNFHNVTAKHEVLLAAGSAVSPTILEYSGIGMKSILEPLGIKTVVDLPVGLNLQDQTTSTVRSRITSAGAGQGQAAWFATFNETFGDYTPKAHELLNTKLEQWAEEAVARGGFHNTTALLIQYENYRDWIVKDNVAYSELFLDTAGEASFDVWDLLPFTRGYVHILDKDPYLRHFAYDPQYFLNELDLLGQAAATQLARNISNSGAMQTYFAGETIPGDNLAYDADLRAWVEYIPYHFRPNYHGVGTCSMMPKEMGGVVDNAARVYGVQGLRVIDGSIPPTQMSSHVMTVFYAMALKIADAVLADYASMQ

SEQ ID NO: 15 - DNA, 1746 bp, synthetic construct
  source 1..1746: mol_type = other DNA
ggtattgaggcttccttgttgactgacccaaaggaggtcgccggtagaactgttgactacatcattgctggtggtggattgactggtttggttgtcgctgccagattgactgagaacccagacatcaccgttttggtcattgagtccggttcttacgaatctgatagaggtcctatcattgaagacttgaacgcttacggtaaaatcttcggatcttccgttgaccacgcttacgagactgtctgccttgccactaacaatagaaccgctttgattagagctggtaacggtttgggtggttctactttggttaacggaggtacttggaccagaccacacaaggctcaagttgactcttgggagaccgtcttcggtaacgaaggttggaattgggattctgtcgcagcttactccttgcaggccgagagagcccgtgctccaaacgctaagcaaatcgccgcaggtcactacttcaacgcctcctgtcacggtattaacggaactgttcacgctggtccaagagacaccggtgacgattactctcctatcgtcaaggccttgatgtccgctgttgaagacagaggtgtcccaactaagaaggacttgtgttgcggagacccacatggtgtttctatgttccctaacaccttgcacccagaccaagtcagatccgatgctgcccgtgaatggttgcttccaaactaccaaagacctaacttgcaggttttgaccggtcaatacgttggtaaggtccttttgtctcaaaacgccactaccccaagagctgttggtgtcgagttcggaactcacaagggtaactttcacaatgttaccgctaaacacgaagtccttttggcagctggttccgctgtttctccaactatcttggagtactctggtatcggaatgaagtccattttggaaccacttggtattaagaccgtcgttgacttgcctgttggtctgaacttgcaagaccagactacctctactgtcagatcccgtattacctccgccggtgctggacagggtcaggctgcctggtttgctactttcaacgagaccttcggtgactacactccaaaggctcacgaattgcttaacaccaaattggaacaatgggctgaggaagccgttgctagaggtggtttccacaacactaccgctcttttgatccaatacgagaactacagagactggattgttaaggataacgtcgcttactctgaattgttcttggacactgccggtgaggcttccttcgacgtctgggacttgctgccattcactagaggatacgttcacatcttggacaaggacccatacttgagacacttcgcttacgatcctcaatacttcttgaacgagttggacttgcttggtcaggctgccgctactcaattggctagaaacatctctaactccggtgccatgcaaacttactttgctggtgaaaccattccaggtgacaacttggcctacgatgctgacttgagagcttgggttgaatacattccataccacttcagacctaactaccatggtgtcggaacctgttctatgatgccaaaggagatgggtggtgtcgttgacaacgccgctagagtttacggtgtccagggattgagagttatcgacggttctatcccacctactcaaatgtcctctcacgttatgaccgtcttctacgctatggctttgaagatcgcagacgctgttttggctgactacgcctccatgcaataa

SEQ ID NO: 16 - protein, 581 aa, synthetic construct
GIEASLLTDPKEVAGRTVDYIIAGGGLTGLVVAARLTENPDITVLVIESGSYESDRGPIIEDLNAYGKIFGSSVDHAYETVCLATNNRTALIRAGNGLGGSTLVNGGTWTRPHKAQVDSWETVFGNEGWNWDSVAAYSLQAERARAPNAKQIAAGHYFNASCHGINGTVHAGPRDTGDDYSPIVKALMSAVEDRGVPTKKDLGCGDPHGVSMFPNTLHEDQVRSDAAREWLLPNYQRPNLSVLTGQYVGKVLLSQNATTPRAVGVEFGTHKGNFHNVTAKHEVLLAAGSAVSPTILEYSGIGMKSILEPLGIKTVVDLPVGLNLQDQTTSTVRSRITPAGAGQGQAAWFATFNETFGDYTPKAHELLNTKLEQWAEEAVARGGFHNTTALLIQYENYRDWIVKDNVAYSELFLDTAGEASFDVWDLLPFTRGYVHILDKDPYLRHFAYDPQYFLNELDLLGQAAATQLARNISNSGAMQTYFAGETIPGDNLAYDADLRAWVEYIPYHFRPNYHGVGTCSMMPKEMGGVVDNAARVYGVQGLRVIDGSIPPTQMSSHVMTVFYAMALKIADAVLADYASMQ

SEQ ID NO: 17 - DNA, 1746 bp, synthetic construct
  source 1..1746: mol_type = other DNA
ggtattgaggcttccttgttgactgacccaaaggaggtcgccggtagaactgttgactacatcattgctggtggtggattgactggtttggttgtcgctgccagattgactgagaacccagacatcaccgttttggtcattgagtccggttcttacgaatctgatagaggtcctatcattgaagacttgaacgcttacggtaaaatcttcggatcttccgttgaccacgcttacgagactgtctgccttgccactaacaatagaaccgctttgattagagctggtaacggtttgggtggttctactttggttaacggaggtacttggaccagaccacacaaggctcaagttgactcttgggagaccgtcttcggtaacgaaggttggaattgggattctgtcgcagcttactccttgcaggccgagagagcccgtgctccaaacgctaagcaaatcgccgcaggtcactacttcaacgcctcctgtcacggtattaacggaactgttcacgctggtccaagagacaccggtgacgattactctcctatcgtcaaggccttgatgtccgctgttgaagacagaggtgtcccaactaagaaggacttgggttgcggagacccacatggtgtttctatgttccctaacaccttgcacgaggaccaagtcagatccgatgctgcccgtgaatggttgcttccaaactaccaaagacctaacttgcaggttttgaccggtcaatacgttggtaaggtccttttgtctcaaaacgccactaccccaagagctgttggtgtcgagttcggaactcacaagggtaactttcacaatgttaccgctaaacacgaagtccttttggcagctggttccgctgtttctccaactatcttggagtactctggtatcggaatgaagtccattttggaaccacttggtattaagaccgtcgttgacttgcctgttggtctgaacttgcaagaccagactacctctactgtcagatcccgtattaccccagccggtgctggacagggtcaggctgcctggtttgctactttcaacgagaccttcggtgactacactccaaaggctcacgaattgcttaacaccaaattggaacaatgggctgaggaagccgttgctagaggtggtttccacaacactaccgctcttttgatccaatacgagaactacagagactggattgttaaggataacgtcgcttactctgaattgttcttggacactgccggtgaggcttccttcgacgtctgggacttgctgccattcactagaggatacgttcacatcttggacaaggacccatacttgagacacttcgcttacgatcctcaatacttcttgaacgagttggacttgcttggtcaggctgccgctactcaattggctagaaacatctctaactccggtgccatgcaaacttactttgctggtgaaaccattccaggtgacaacttggcctacgatgctgacttgagagcttgggttgaatacattccataccacttcagacctaactaccatggtgtcggaacctgttctatgatgccaaaggagatgggtggtgtcgttgacaacgccgctagagtttacggtgtccagggattgagagttatcgacggttctatcccacctactcaaatgtcctctcacgttatgaccgtcttctacgctatggctttgaagatcgcagacgctgttttggctgactacgcctccatgcaataa

SEQ ID NO: 18 - protein, 581 aa, synthetic construct
GIEASLLTDPKEVAGRTVDYIIAGGGLTGLVVAARLTENPDITVLVIESGSYESDRGPIIEDLNAYGKIFGSSVDHAYETVCLATNNRTALIRAGNGLGGSTLVNGGTWTRPHKAQVDSWETVFGNEGWNWDSVAAYSLQAERARAPNAKQIAAGHYFNASCHGINGTVHAGPRDTGDDYSPIVKALMSAVEDRGVPTKKDLGCGDPHGVSMFPNTLHEDQVRSDAAREWLLPNYQRPNLSVLTGQYVGKVLLSQNATTPRAVGVEFGTHKGNFHNVTAKHEVLLAAGSAVSPTILEYSGIGMKSILEPLGIKTVVDLPVGLNLQDQTTSTVRSRITSAGAGQGQAAWFATFNETFGDYTPKAHELLNTKLEQWAEEAVARGGFHNTTALLIQYENYRDWIVKDNVAYSELFLDTAGEISFDVWDLLPFTRGYVHILDKDPYLRHFAYDPQYFLNELDLLGQAAATQLARNISNSGAMQTYFAGETIPGDNLAYDADLRAWVEYIPYHFRPNYHGVGTCSMMPKEMGGVVDNAARVYGVQGLRVIDGSIPPTQMSSHVMTVFYAMALKIADAVLADYASMQ

SEQ ID NO: 19 - DNA, 1746 bp, synthetic construct
  source 1..1746: mol_type = other DNA
ggtattgaggcttccttgttgactgacccaaaggaggtcgccggtagaactgttgactacatcattgctggtggtggattgactggtttggttgtcgctgccagattgactgagaacccagacatcaccgttttggtcattgagtccggttcttacgaatctgatagaggtcctatcattgaagacttgaacgcttacggtaaaatcttcggatcttccgttgaccacgcttacgagactgtctgccttgccactaacaatagaaccgctttgattagagctggtaacggtttgggtggttctactttggttaacggaggtacttggaccagaccacacaaggctcaagttgactcttgggagaccgtcttcggtaacgaaggttggaattgggattctgtcgcagcttactccttgcaggccgagagagcccgtgctccaaacgctaagcaaatcgccgcaggtcactacttcaacgcctcctgtcacggtattaacggaactgttcacgctggtccaagagacaccggtgacgattactctcctatcgtcaaggccttgatgtccgctgttgaagacagaggtgtcccaactaagaaggacttgggttgcggagacccacatggtgtttctatgttccctaacaccttgcacgaggaccaagtcagatccgatgctgcccgtgaatggttgcttccaaactaccaaagacctaacttgcaggttttgaccggtcaatacgttggtaaggtccttttgtctcaaaacgccactaccccaagagctgttggtgtcgagttcggaactcacaagggtaactttcacaatgttaccgctaaacacgaagtccttttggcagctggttccgctgtttctccaactatcttggagtactctggtatcggaatgaagtccattttggaaccacttggtattaagaccgtcgttgacttgcctgttggtctgaacttgcaagaccagactacctctactgtcagatcccgtattacctccgccggtgctggacagggtcaggctgcctggtttgctactttcaacgagaccttcggtgactacactccaaaggctcacgaattgcttaacaccaaattggaacaatgggctgaggaagccgttgctagaggtggtttccacaacactaccgctcttttgatccaatacgagaactacagagactggattgttaaggataacgtcgcttactctgaattgttcttggacactgccggtgagatctccttcgacgtctgggacttgctgccattcactagaggatacgttcacatcttggacaaggacccatacttgagacacttcgcttacgatcctcaatacttcttgaacgagttggacttgcttggtcaggctgccgctactcaattggctagaaacatctctaactccggtgccatgcaaacttactttgctggtgaaaccattccaggtgacaacttggcctacgatgctgacttgagagcttgggttgaatacattccataccacttcagacctaactaccatggtgtcggaacctgttctatgatgccaaaggagatgggtggtgtcgttgacaacgccgctagagtttacggtgtccagggattgagagttatcgacggttctatcccacctactcaaatgtcctctcacgttatgaccgtcttctacgctatggctttgaagatcgcagacgctgttttggctgactacgcctccatgcaataa

SEQ ID NO: 20 - protein, 581 aa, synthetic construct
GIEASLLTDPKEVAGRTVDYIIAGGGLTGLVVAARLTENPDITVLVIESGSYESDRGPIIEDLNAYGKIFGSSVDHAYETVCLATNNRTALIRAGNGLGGSTLVNGGTWTRPHKAQVDSWETVFGNEGWNWDSVAAYSLQAERARAPNAKQIAAGHYFNASCHGINGTVHAGPRDTGDDYSPIVKALMSAVEDRGVPTKKDLCCGDPHGVSMFPNTLHEDQVRSDAAREWLLPNYQRPNLSVLTGQYVGKVLLSQNATTPRAVGVEFGTHKGNFHNVTAKHEVLLAAGSAVSPTILEYSGIGMKSILEPLGIKTVVDLPVGLNLQDQTTSTVRSRITSAGAGQGQAAWFATFNETFGDYTPKAHELLNTKLEQWAEEAVARGGFHNTTALLIQYENYRDWIVKDNVAYSELFLDTAGEISFDVWDLLPFTRGYVHILDKDPYLRHFAYDPQYFLNELDLLGQAAATQLARNISNSGAMQTYFAGETIPGDNLAYDADLRAWVEYIPYHFRPNYHGVGTCSMMPKEMGGVVDNAARVYGVQGLRVIDGSIPPTQMSSHVMTVFYAMALKIADAVLADYASMQ

SEQ ID NO: 21 - DNA, 1746 bp, synthetic construct
  source 1..1746: mol_type = other DNA
ggtattgaggcttccttgttgactgacccaaaggaggtcgccggtagaactgttgactacatcattgctggtggtggattgactggtttggttgtcgctgccagattgactgagaacccagacatcaccgttttggtcattgagtccggttcttacgaatctgatagaggtcctatcattgaagacttgaacgcttacggtaaaatcttcggatcttccgttgaccacgcttacgagactgtctgccttgccactaacaatagaaccgctttgattagagctggtaacggtttgggtggttctactttggttaacggaggtacttggaccagaccacacaaggctcaagttgactcttgggagaccgtcttcggtaacgaaggttggaattgggattctgtcgcagcttactccttgcaggccgagagagcccgtgctccaaacgctaagcaaatcgccgcaggtcactacttcaacgcctcctgtcacggtattaacggaactgttcacgctggtccaagagacaccggtgacgattactctcctatcgtcaaggccttgatgtccgctgttgaagacagaggtgtcccaactaagaaggacttgtgttgcggagacccacatggtgtttctatgttccctaacaccttgcacgaggaccaagtcagatccgatgctgcccgtgaatggttgcttccaaactaccaaagacctaacttgcaggttttgaccggtcaatacgttggtaaggtccttttgtctcaaaacgccactaccccaagagctgttggtgtcgagttcggaactcacaagggtaactttcacaatgttaccgctaaacacgaagtccttttggcagctggttccgctgtttctccaactatcttggagtactctggtatcggaatgaagtccattttggaaccacttggtattaagaccgtcgttgacttgcctgttggtctgaacttgcaagaccagactacctctactgtcagatcccgtattacctccgccggtgctggacagggtcaggctgcctggtttgctactttcaacgagaccttcggtgactacactccaaaggctcacgaattgcttaacaccaaattggaacaatgggctgaggaagccgttgctagaggtggtttccacaacactaccgctcttttgatccaatacgagaactacagagactggattgttaaggataacgtcgcttactctgaattgttcttggacactgccggtgagatctccttcgacgtctgggacttgctgccattcactagaggatacgttcacatcttggacaaggacccatacttgagacacttcgcttacgatcctcaatacttcttgaacgagttggacttgcttggtcaggctgccgctactcaattggctagaaacatctctaactccggtgccatgcaaacttactttgctggtgaaaccattccaggtgacaacttggcctacgatgctgacttgagagcttgggttgaatacattccataccacttcagacctaactaccatggtgtcggaacctgttctatgatgccaaaggagatgggtggtgtcgttgacaacgccgctagagtttacggtgtccagggattgagagttatcgacggttctatcccacctactcaaatgtcctctcacgttatgaccgtcttctacgctatggctttgaagatcgcagacgctgttttggctgactacgcctccatgcaataa

SEQ ID NO: 22 - protein, 581 aa, synthetic construct
GIEASLLTDPKEVAGRTVDYIIAGGGLTGLVVAARLTENPDITVLVIESGSYESDRGPIIEDLNAYGKIFGSSVDHAYETVCLATNNRTALIRAGNGLGGSTLVNGGTWTRPHKAQVDSWETVFGNEGWNWDSVAAYSLQAERARAPNAKQIAAGHYFNASCHGINGTVHAGPRDTGDDYSPIVKALMSAVEDRGVPTKKDLGCGDPHGVSMFPNTLHEDQVRSDAAREWLLPNYQRPNLSVLTGQYVGKVLLSQNATTPRAVGVEFGTHKGNFHNVTAKHEVLLAAGSAVSPTILEYSGIGMKSILEPLGIKTVVDLPVGLNLQDQTTSTVRSRITPAGAGQGQAAWFATFNETFGDYTPKAHELLNTKLEQWAEEAVARGGFHNTTALLIQYENYRDWIVKDNVAYSELFLDTAGEISFDVWDLLPFTRGYVHILDKDPYLRHFAYDPQYFLNELDLLGQAAATQLARNISNSGAMQTYFAGETIPGDNLAYDADLRAWVEYIPYHFRPNYHGVGTCSMMPKEMGGVVDNAARVYGVQGLRVIDGSIPPTQMSSHVMTVFYAMALKIADAVLADYASMQ

SEQ ID NO: 23 - DNA, 1746 bp, synthetic construct
  source 1..1746: mol_type = other DNA
ggtattgaggcttccttgttgactgacccaaaggaggtcgccggtagaactgttgactacatcattgctggtggtggattgactggtttggttgtcgctgccagattgactgagaacccagacatcaccgttttggtcattgagtccggttcttacgaatctgatagaggtcctatcattgaagacttgaacgcttacggtaaaatcttcggatcttccgttgaccacgcttacgagactgtctgccttgccactaacaatagaaccgctttgattagagctggtaacggtttgggtggttctactttggttaacggaggtacttggaccagaccacacaaggctcaagttgactcttgggagaccgtcttcggtaacgaaggttggaattgggattctgtcgcagcttactccttgcaggccgagagagcccgtgctccaaacgctaagcaaatcgccgcaggtcactacttcaacgcctcctgtcacggtattaacggaactgttcacgctggtccaagagacaccggtgacgattactctcctatcgtcaaggccttgatgtccgctgttgaagacagaggtgtcccaactaagaaggacttgggttgcggagacccacatggtgtttctatgttccctaacaccttgcacgaggaccaagtcagatccgatgctgcccgtgaatggttgcttccaaactaccaaagacctaacttgcaggttttgaccggtcaatacgttggtaaggtccttttgtctcaaaacgccactaccccaagagctgttggtgtcgagttcggaactcacaagggtaactttcacaatgttaccgctaaacacgaagtccttttggcagctggttccgctgtttctccaactatcttggagtactctggtatcggaatgaagtccattttggaaccacttggtattaagaccgtcgttgacttgcctgttggtctgaacttgcaagaccagactacctctactgtcagatcccgtattaccccagccggtgctggacagggtcaggctgcctggtttgctactttcaacgagaccttcggtgactacactccaaaggctcacgaattgcttaacaccaaattggaacaatgggctgaggaagccgttgctagaggtggtttccacaacactaccgctcttttgatccaatacgagaactacagagactggattgttaaggataacgtcgcttactctgaattgttcttggacactgccggtgagatctccttcgacgtctgggacttgctgccattcactagaggatacgttcacatcttggacaaggacccatacttgagacacttcgcttacgatcctcaatacttcttgaacgagttggacttgcttggtcaggctgccgctactcaattggctagaaacatctctaactccggtgccatgcaaacttactttgctggtgaaaccattccaggtgacaacttggcctacgatgctgacttgagagcttgggttgaatacattccataccacttcagacctaactaccatggtgtcggaacctgttctatgatgccaaaggagatgggtggtgtcgttgacaacgccgctagagtttacggtgtccagggattgagagttatcgacggttctatcccacctactcaaatgtcctctcacgttatgaccgtcttctacgctatggctttgaagatcgcagacgctgttttggctgactacgcctccatgcaataa

SEQ ID NO: 24 - protein, 581 aa, synthetic construct
GIEASLLTDPKEVAGRTVDYIIAGGGLTGLVVAARLTENPDITVLVIESGSYESDRGPIIEDLNAYGKIFGSSVDHAYETVCLATNNRTALIRAGNGLGGSTLVNGGTWTRPHKAQVDSWETVFGNEGWNWDSVAAYSLQAERARAPNAKQIAAGHYFNASCHGINGTVHAGPRDTGDDYSPIVKALMSAVENRGVPTKKDLGCGDPHGVSMFPNTLHEDQVRSDAAREWLLPNYQRPNLSVLTGQYVGKVLLSQNATTPRAVGVEFGTHKGNFHNVTAKHEVLLAAGSAVSPTILEYSGIGMKSILEPLGIKTVVDLPVGLNLQDQTTSTVRSRITSAGAGQGQAAWFATFNETFGDYTPKAHELLNTKLEQWAEEAVARGGFHNTTALLIQYENYRDWIVKDNVAYSELFLDTAGEISFDVWDLLPFTRGYVHILDKDPYLRHFAYDPQYFLNELDLLGQAAATQLARNISNSGAMQTYFAGETIPGDNLAYDANLRAWVEYIPYHFRPNYHGVGTCSMMPKEMGGVVDNAARVYGVQGLRVIDGSIPPTQMSSHVMTVFYAMALKIADAVLADYASMQ

SEQ ID NO: 25 - DNA, 1746 bp, synthetic construct
  source 1..1746: mol_type = other DNA
ggtattgaggcttccttgttgactgacccaaaggaggtcgccggtagaactgttgactacatcattgctggtggtggattgactggtttggttgtcgctgccagattgactgagaacccagacatcaccgttttggtcattgagtccggttcttacgaatctgatagaggtcctatcattgaagacttgaacgcttacggtaaaatcttcggatcttccgttgaccacgcttacgagactgtctgccttgccactaacaatagaaccgctttgattagagctggtaacggtttgggtggttctactttggttaacggaggtacttggaccagaccacacaaggctcaagttgactcttgggagaccgtcttcggtaacgaaggttggaattgggattctgtcgcagcttactccttgcaggccgagagagcccgtgctccaaacgctaagcaaatcgccgcaggtcactacttcaacgcctcctgtcacggtattaacggaactgttcacgctggtccaagagacaccggtgacgattactctcctatcgtcaaggccttgatgtccgctgttgaaaacagaggtgtcccaactaagaaggacttgggttgcggagacccacatggtgtttctatgttccctaacaccttgcacgaggaccaagtcagatccgatgctgcccgtgaatggttgcttccaaactaccaaagacctaacttgcaggttttgaccggtcaatacgttggtaaggtccttttgtctcaaaacgccactaccccaagagctgttggtgtcgagttcggaactcacaagggtaactttcacaatgttaccgctaaacacgaagtccttttggcagctggttccgctgtttctccaactatcttggagtactctggtatcggaatgaagtccattttggaaccacttggtattaagaccgtcgttgacttgcctgttggtctgaacttgcaagaccagactacctctactgtcagatcccgtattacctccgccggtgctggacagggtcaggctgcctggtttgctactttcaacgagaccttcggtgactacactccaaaggctcacgaattgcttaacaccaaattggaacaatgggctgaggaagccgttgctagaggtggtttccacaacactaccgctcttttgatccaatacgagaactacagagactggattgttaaggataacgtcgcttactctgaattgttcttggacactgccggtgagatctccttcgacgtctgggacttgctgccattcactagaggatacgttcacatcttggacaaggacccatacttgagacacttcgcttacgatcctcaatacttcttgaacgagttggacttgcttggtcaggctgccgctactcaattggctagaaacatctctaactccggtgccatgcaaacttactttgctggtgaaaccattccaggtgacaacttggcctacgatgctaacttgagagcttgggttgaatacattccataccacttcagacctaactaccatggtgtcggaacctgttctatgatgccaaaggagatgggtggtgtcgttgacaacgccgctagagtttacggtgtccagggattgagagttatcgacggttctatcccacctactcaaatgtcctctcacgttatgaccgtcttctacgctatggctttgaagatcgcagacgctgttttggctgactacgcctccatgcaataa

SEQ ID NO: 26 - protein, 581 aa, synthetic construct
GIEDSLLTDPKEVAGRTVDYIIAGGGLTGLVVAARLTENPDITVLVIESGSYESDRGPIIEDLNAYGKIFGSSVDHAYETVCLATNNRTALIRAGNGLGGSTLVNGGTWTRPHKAQVDSWETVFGNEGWNWDSVAAYSLQAERARAPNAKQIAAGHYFNASCHGINGTVHAGPRDTGDDYSPIVKALMSAVEDRGVPTKKDLGCGDPHGVSMFPNTLHEDQVRSDAAREWLLPNYQRPNLSVLTGQYVGKVLLSQNATTPRAVGVEFGTHKGNFHNVTAKHEVLLAAGSAVSPTILEYSGIGMKSILEPLGIKTVVDLPVGLNLQDQTTSTVRSRITSAGAGQGQAAWFATFNETFGDYTPKAHELLNTKLEQWAEEAVARGGFHNTTALLIQYENYRDWIVKDNVAYSELFLDTAGEISFDVWDLLPFTRGYVHILDKDPYLRHFAYDPQYFLNELDLLGQAAATQLAREISNSGAMQTYFAGETIPGDNLAYDADLRAWVEYIPYHFRPNYHGVGTCSMMPKEMGGVVDNAARVYGVQGLRVIDGSIPPTQMSSHVMTVFYAMALKIADAVLADYASMQ

SEQ ID NO: 27 - DNA, 1746 bp, synthetic construct
  source 1..1746: mol_type = other DNA
ggtattgaggattccttgttgactgacccaaaggaggtcgccggtagaactgttgactacatcattgctggtggtggattgactggtttggttgtcgctgccagattgactgagaacccagacatcaccgttttggtcattgagtccggttcttacgaatctgatagaggtcctatcattgaagacttgaacgcttacggtaaaatcttcggatcttccgttgaccacgcttacgagactgtctgccttgccactaacaatagaaccgctttgattagagctggtaacggtttgggtggttctactttggttaacggaggtacttggaccagaccacacaaggctcaagttgactcttgggagaccgtcttcggtaacgaaggttggaattgggattctgtcgcagcttactccttgcaggccgagagagcccgtgctccaaacgctaagcaaatcgccgcaggtcactacttcaacgcctcctgtcacggtattaacggaactgttcacgctggtccaagagacaccggtgacgattactctcctatcgtcaaggccttgatgtccgctgttgaagacagaggtgtcccaactaagaaggacttgggttgcggagacccacatggtgtttctatgttccctaacaccttgcacgaggaccaagtcagatccgatgctgcccgtgaatggttgcttccaaactaccaaagacctaacttgcaggttttgaccggtcaatacgttggtaaggtccttttgtctcaaaacgccactaccccaagagctgttggtgtcgagttcggaactcacaagggtaactttcacaatgttaccgctaaacacgaagtccttttggcagctggttccgctgtttctccaactatcttggagtactctggtatcggaatgaagtccattttggaaccacttggtattaagaccgtcgttgacttgcctgttggtctgaacttgcaagaccagactacctctactgtcagatcccgtattacctccgccggtgctggacagggtcaggctgcctggtttgctactttcaacgagaccttcggtgactacactccaaaggctcacgaattgcttaacaccaaattggaacaatgggctgaggaagccgttgctagaggtggtttccacaacactaccgctcttttgatccaatacgagaactacagagactggattgttaaggataacgtcgcttactctgaattgttcttggacactgccggtgagatctccttcgacgtctgggacttgctgccattcactagaggatacgttcacatcttggacaaggacccatacttgagacacttcgcttacgatcctcaatacttcttgaacgagttggacttgcttggtcaggctgccgctactcaattggctagagaaatctctaactccggtgccatgcaaacttactttgctggtgaaaccattccaggtgacaacttggcctacgatgctgacttgagagcttgggttgaatacattccataccacttcagacctaactaccatggtgtcggaacctgttctatgatgccaaaggagatgggtggtgtcgttgacaacgccgctagagtttacggtgtccagggattgagagttatcgacggttctatcccacctactcaaatgtcctctcacgttatgaccgtcttctacgctatggctttgaagatcgcagacgctgttttggctgactacgcctccatgcaataa

SEQ ID NO: 28 - protein, 581 aa, synthetic construct
GIEDSLLTDPKEVAGRTVDYIIAGGGLTGLVVAARLTENPDITVLVIESGSYESDRGPIIEDLNAYGKIFGSSVDHAYETVCLATNNRTALIRAGNGLGGSTLVNGGTWTRPHKAQVDSWETVFGNEGWNWDSVAAYSLQAERARAPNAKQIAAGHYFNASCHGINGTVHAGPRDTGDDYSPIVKALMSAVENRGVPTKKDLGCGDPHGVSMFPNTLHEDQVRSDAAREWLLPNYQRPNLSVLTGQYVGKVLLSQNATTPRAVGVEFGTHKGNFHNVTAKHEVLLAAGSAVSPTILEYSGIGMKSILEPLGIKTVVDLPVGLNLQDQTTSTVRSRITSAGAGQGQAAWFATFNETFGDYTPKAHELLNTKLEQWAEEAVARGGFHNTTALLIQYENYRDWIVKDNVAYSELFLDTAGEISFDVWDLLPFTRGYVHILDKDPYLRHFAYDPQYFLNELDLLGQAAATQLAREISNSGAMQTYFAGETIPGDNLAYDANLRAWVEYIPYHFRPNYHGVGTCSMMPKEMGGVVDNAARVYGVQGLRVIDGSIPPTQMSSHVMTVFYAMALKIADAVLADYASMQ

SEQ ID NO: 29 - DNA, 1746 bp, synthetic construct
  source 1..1746: mol_type = other DNA
ggtattgaggattccttgttgactgacccaaaggaggtcgccggtagaactgttgactacatcattgctggtggtggattgactggtttggttgtcgctgccagattgactgagaacccagacatcaccgttttggtcattgagtccggttcttacgaatctgatagaggtcctatcattgaagacttgaacgcttacggtaaaatcttcggatcttccgttgaccacgcttacgagactgtctgccttgccactaacaatagaaccgctttgattagagctggtaacggtttgggtggttctactttggttaacggaggtacttggaccagaccacacaaggctcaagttgactcttgggagaccgtcttcggtaacgaaggttggaattgggattctgtcgcagcttactccttgcaggccgagagagcccgtgctccaaacgctaagcaaatcgccgcaggtcactacttcaacgcctcctgtcacggtattaacggaactgttcacgctggtccaagagacaccggtgacgattactctcctatcgtcaaggccttgatgtccgctgttgaaaacagaggtgtcccaactaagaaggacttgggttgcggagacccacatggtgtttctatgttccctaacaccttgcacgaggaccaagtcagatccgatgctgcccgtgaatggttgcttccaaactaccaaagacctaacttgcaggttttgaccggtcaatacgttggtaaggtccttttgtctcaaaacgccactaccccaagagctgttggtgtcgagttcggaactcacaagggtaactttcacaatgttaccgctaaacacgaagtccttttggcagctggttccgctgtttctccaactatcttggagtactctggtatcggaatgaagtccattttggaaccacttggtattaagaccgtcgttgacttgcctgttggtctgaacttgcaagaccagactacctctactgtcagatcccgtattacctccgccggtgctggacagggtcaggctgcctggtttgctactttcaacgagaccttcggtgactacactccaaaggctcacgaattgcttaacaccaaattggaacaatgggctgaggaagccgttgctagaggtggtttccacaacactaccgctcttttgatccaatacgagaactacagagactggattgttaaggataacgtcgcttactctgaattgttcttggacactgccggtgagatctccttcgacgtctgggacttgctgccattcactagaggatacgttcacatcttggacaaggacccatacttgagacacttcgcttacgatcctcaatacttcttgaacgagttggacttgcttggtcaggctgccgctactcaattggctagagaaatctctaactccggtgccatgcaaacttactttgctggtgaaaccattccaggtgacaacttggcctacgatgctaacttgagagcttgggttgaatacattccataccacttcagacctaactaccatggtgtcggaacctgttctatgatgccaaaggagatgggtggtgtcgttgacaacgccgctagagtttacggtgtccagggattgagagttatcgacggttctatcccacctactcaaatgtcctctcacgttatgaccgtcttctacgctatggctttgaagatcgcagacgctgttttggctgactacgcctccatgcaataa

SEQ ID NO: 30 - DNA, 30 bp, synthetic construct
  source 1..30: mol_type = other DNA
ggtattgaggcttccttgttgactgaccca

SEQ ID NO: 31 - DNA, 30 bp, synthetic construct
  source 1..30: mol_type = other DNA
ttgcatggaggcgtagtcagccaaaacagc

SEQ ID NO: 32 - DNA, 30 bp, synthetic construct
  source 1..30: mol_type = other DNA
actaagaaggacttgtgttgcggagaccca

SEQ ID NO: 33 - DNA, 30 bp, synthetic construct
  source 1..30: mol_type = other DNA
atgtgggtctccgcaacacaagtccttctt

SEQ ID NO: 34 - DNA, 30 bp, synthetic construct
  source 1..30: mol_type = other DNA
cctaacaccttgcacccagaccaagtcaga

SEQ ID NO: 35 - DNA, 30 bp, synthetic construct
  source 1..30: mol_type = other DNA
ggatctgacttggtctgggtgcaaggtgtt

SEQ ID NO: 36 - DNA, 30 bp, synthetic construct
  source 1..30: mol_type = other DNA
agatcccgtattaccccagccggtgctgga

SEQ ID NO: 37 - DNA, 30 bp, synthetic construct
  source 1..30: mol_type = other DNA
ctgtccagcaccggctggggtaatacggga

SEQ ID NO: 38 - DNA, 30 bp, synthetic construct
  source 1..30: mol_type = other DNA
ttcggtgactacactccaaaggctcacgaa

SEQ ID NO: 39 - DNA, 30 bp, synthetic construct
  source 1..30: mol_type = other DNA
caattcgtgagcctttggagtgtagtcacc

SEQ ID NO: 40 - DNA, 30 bp, synthetic construct
  source 1..30: mol_type = other DNA
gacactgccggtgagatctccttcgacgtc

SEQ ID NO: 41 - DNA, 30 bp, synthetic construct
  source 1..30: mol_type = other DNA
ccagacgtcgaaggagatctcaccggcagt